European Patent Specification EP 3 891 285 B1, published June 24, 2026. Title: APTAMERS AND THE USE THEREOF IN THE TREATMENT OF CANCER. Applicant: Fundación para la Investigación Biomédica del Hospital Ramón y Cajal. The sequence listing filed with the application follows.

SEQUENCE LISTING (5 sequences)

SEQ ID NO: 1 - DNA, 48 bp, Artificial Sequence
  apMNK2FT
  misc_feature (1)..(48)
tttttggggtgggcgggcgggggtgggggtggtatggcgcgttggccc

SEQ ID NO: 2 - DNA, 18 bp, Artificial Sequence
  apMNKQ1
  misc_feature (1)..(18)
tggggtgggcgggcgggg

SEQ ID NO: 3 - DNA, 29 bp, Artificial Sequence
  apMNKQ2
  misc_feature (1)..(29)
tggggtgggcgggcgggggtgggggtggt

SEQ ID NO: 4 - DNA, 13 bp, Artificial Sequence
  apMNKQ3
  misc_feature (1)..(13)
gggtgggggtggt

SEQ ID NO: 5 - DNA, 22 bp, Artificial Sequence
  apMNKQ4
  misc_feature (1)..(22)
gggtggtatggcgcgttggccc